European Patent Application EP 4 533 942 A1, published April 9, 2025. Title: Animal fibers derived from a genetically engineered animal. Applicant: OPTAGE INC. The sequence listing filed with the application follows.

SEQUENCE LISTING (108 sequences)

SEQ ID NO: 1 - RNA, 20 nt, synthetic construct
  misc_feature 1..20: note = Krt71 crRNA1
  source 1..20: mol_type = other RNA
cctaccgggcaggaggcaaa

SEQ ID NO: 2 - RNA, 20 nt, synthetic construct
  misc_feature 1..20: note = Krt71 crRNA2
  source 1..20: mol_type = other RNA
agcgggaagaacggaggttt

SEQ ID NO: 3 - RNA, 20 nt, synthetic construct
  misc_feature 1..20: note = Krt71 crRNA3
  source 1..20: mol_type = other RNA
acctgatggataccgccagg

SEQ ID NO: 4 - RNA, 20 nt, synthetic construct
  misc_feature 1..20: note = Krt72 crRNA1
  source 1..20: mol_type = other RNA
gtcatctcaggcaggctcag

SEQ ID NO: 5 - RNA, 20 nt, synthetic construct
  misc_feature 1..20: note = Krt72 crRNA2
  source 1..20: mol_type = other RNA
agaagcctgttctgtgtggg

SEQ ID NO: 6 - RNA, 20 nt, synthetic construct
  misc_feature 1..20: note = Krt72 crRNA3
  source 1..20: mol_type = other RNA
cgggatagagggtcaactgg

SEQ ID NO: 7 - RNA, 20 nt, synthetic construct
  misc_feature 1..20: note = Krt73 crRNA1
  source 1..20: mol_type = other RNA
tcttaccgggcagccggcaa

SEQ ID NO: 8 - RNA, 20 nt, synthetic construct
  misc_feature 1..20: note = Krt73 crRNA2
  source 1..20: mol_type = other RNA
agcgggcgcacagggggata

SEQ ID NO: 9 - RNA, 20 nt, synthetic construct
  misc_feature 1..20: note = Krt73 crRNA3
  source 1..20: mol_type = other RNA
aatccatccttgtgcctgcc

SEQ ID NO: 10 - RNA, 20 nt, synthetic construct
  misc_feature 1..20: note = Krt74 crRNA1
  source 1..20: mol_type = other RNA
gattccctccaagactgtag

SEQ ID NO: 11 - RNA, 20 nt, synthetic construct
  misc_feature 1..20: note = Krt74 crRNA2
  source 1..20: mol_type = other RNA
agctttggatatgggtatgg

SEQ ID NO: 12 - RNA, 20 nt, synthetic construct
  misc_feature 1..20: note = Krt74 crRNA3
  source 1..20: mol_type = other RNA
tctgtctgggggcatctacc

SEQ ID NO: 13 - RNA, 20 nt, synthetic construct
  misc_feature 1..20: note = KAP8-1 crRNA1
  source 1..20: mol_type = other RNA
gtcttcccaggatgctactg

SEQ ID NO: 14 - RNA, 20 nt, synthetic construct
  misc_feature 1..20: note = KAP8-1 crRNA2
  source 1..20: mol_type = other RNA
cagccaacactgtaccccag

SEQ ID NO: 15 - RNA, 20 nt, synthetic construct
  misc_feature 1..20: note = KAP8-1 crRNA3
  source 1..20: mol_type = other RNA
ggtagcacctactctccagt

SEQ ID NO: 16 - RNA, 20 nt, synthetic construct
  misc_feature 1..20: note = KAP8-2 crRNA1
  source 1..20: mol_type = other RNA
gtagctgccgtagtagctca

SEQ ID NO: 17 - RNA, 20 nt, synthetic construct
  misc_feature 1..20: note = KAP8-2 crRNA2
  source 1..20: mol_type = other RNA
ggctctggcatccgaggctt

SEQ ID NO: 18 - RNA, 20 nt, synthetic construct
  misc_feature 1..20: note = KAP8-2 crRNA3
  source 1..20: mol_type = other RNA
ggaggttacggatatggatc

SEQ ID NO: 19 - RNA, 20 nt, synthetic construct
  misc_feature 1..20: note = Tyr crRNA1
  source 1..20: mol_type = other RNA
tgccaacaagttcttagagg

SEQ ID NO: 20 - RNA, 20 nt, synthetic construct
  misc_feature 1..20: note = Tyr crRNA2
  source 1..20: mol_type = other RNA
ggtcatccacccctttgaag

SEQ ID NO: 21 - RNA, 20 nt, synthetic construct
  misc_feature 1..20: note = Tyr crRNA3
  source 1..20: mol_type = other RNA
cagtgctcaggcaacttcat

SEQ ID NO: 22 - RNA, 20 nt, synthetic construct
  misc_feature 1..20: note = Fgf5 crRNA1
  source 1..20: mol_type = other RNA
cccaagcgctgtggatcagg

SEQ ID NO: 23 - RNA, 20 nt, synthetic construct
  misc_feature 1..20: note = Fgf5 crRNA2
  source 1..20: mol_type = other RNA
acgtcgcgctacttctgccc

SEQ ID NO: 24 - RNA, 20 nt, synthetic construct
  misc_feature 1..20: note = Fgf5 crRNA3
  source 1..20: mol_type = other RNA
gtttccagtggagcccttcg

SEQ ID NO: 25 - DNA, 54 bp, synthetic construct
  misc_feature 1..54: note = Krt71_Miseq_Fw
  source 1..54: mol_type = other DNA
tcgtcggcagcgtcagatgtgtataagagacagatctaccttcctcctgcacct

SEQ ID NO: 26 - DNA, 55 bp, synthetic construct
  misc_feature 1..55: note = Krt71_Miseq_Rv
  source 1..55: mol_type = other DNA
gtctcgtgggctcggagatgtgtataagagacattgttcagagccttgatctgct

SEQ ID NO: 27 - DNA, 22 bp, synthetic construct
  misc_feature 1..22: note = Krt72 N-Fw
  source 1..22: mol_type = other DNA
aattagctgactccatcctgcc

SEQ ID NO: 28 - DNA, 22 bp, synthetic construct
  misc_feature 1..22: note = Krt72 N-Rv
  source 1..22: mol_type = other DNA
ccttgatctgctccctctcttg

SEQ ID NO: 29 - DNA, 55 bp, synthetic construct
  misc_feature 1..55: note = Krt73_Miseq_Fw
  source 1..55: mol_type = other DNA
tcgtcggcagcgtcagatgtgtataagagacagctgtctgtggcttcttcaggat

SEQ ID NO: 30 - DNA, 55 bp, synthetic construct
  misc_feature 1..55: note = Krt73_Miseq_Rv
  source 1..55: mol_type = other DNA
gtctcgtgggctcggagatgtgtataagagacagcgaatttgttgttcagagcct

SEQ ID NO: 31 - DNA, 55 bp, synthetic construct
  misc_feature 1..55: note = Krt74_Miseq_Fw
  source 1..55: mol_type = other DNA
tcgtcggcagcgtcagatgtgtataagagacaggttggcaactgaacttcaggtc

SEQ ID NO: 32 - DNA, 55 bp, synthetic construct
  misc_feature 1..55: note = Krt74_Miseq_Rv
  source 1..55: mol_type = other DNA
gtctcgtgggctcggagatgtgtataagagacaacttgtcgttcagagccttgat

SEQ ID NO: 33 - DNA, 22 bp, synthetic construct
  misc_feature 1..22: note = KAP8-1 Fw
  source 1..22: mol_type = other DNA
aagaccaagcgcttttgaagtc

SEQ ID NO: 34 - DNA, 22 bp, synthetic construct
  misc_feature 1..22: note = KAP8-1 Rv
  source 1..22: mol_type = other DNA
aggtgtcacaaagccttcatga

SEQ ID NO: 35 - DNA, 57 bp, synthetic construct
  misc_feature 1..57: note = KAP8-1-Miseq_Fw
  source 1..57: mol_type = other DNA
tcgtcggcagcgtcagatgtgtataagagacagaagaatgaaaatgagggccttgtg

SEQ ID NO: 36 - DNA, 56 bp, synthetic construct
  misc_feature 1..56: note = KAP8-1-Miseq_Rv
  source 1..56: mol_type = other DNA
gtctcgtgggctcggagatgtgtataagagacagaggtgtcacaaagccttcatga

SEQ ID NO: 37 - DNA, 56 bp, synthetic construct
  misc_feature 1..56: note = KAP8-2_Miseq_Fw
  source 1..56: mol_type = other DNA
tcgtcggcagcgtcagatgtgtataagagacagacaacggaagggtatgttcatga

SEQ ID NO: 38 - DNA, 60 bp, synthetic construct
  misc_feature 1..60: note = KAP8-2_Miseq_Rv
  source 1..60: mol_type = other DNA
gtctcgtgggctcggagatgtgtataagagacatttcttcttgacttgattcacagtcag

SEQ ID NO: 39 - DNA, 20 bp, synthetic construct
  misc_feature 1..20: note = Tyr Fw
  source 1..20: mol_type = other DNA
ccaggggttgctggaaaaga

SEQ ID NO: 40 - DNA, 23 bp, synthetic construct
  misc_feature 1..23: note = Tyr Rv
  source 1..23: mol_type = other DNA
tcttttcggagacactcaaatca

SEQ ID NO: 41 - DNA, 20 bp, synthetic construct
  misc_feature 1..20: note = Fgf5 Fw
  source 1..20: mol_type = other DNA
gaggctatgtccaccctgtg

SEQ ID NO: 42 - DNA, 20 bp, synthetic construct
  misc_feature 1..20: note = Fgf5 Rv
  source 1..20: mol_type = other DNA
gtccctcccagaacaggttt

SEQ ID NO: 43 - DNA, 419 bp, synthetic construct
  misc_feature 1..419: note = Krt71 WT
  source 1..419: mol_type = other DNA
atgagccgccaattcacctgcaagtctggagccagcaacaggggcttcagtggttgctccgcagtgctctctgggggaagctcatcctcctaccgggcaggaggcaaagggctcagcgggggctttggcagtcggagtctctacagcctgggaggtggcaggagcatcactcttaacatggctagtggcagcgggaagaacggaggttttggatttggccggaaccgagccagtggctttgccggaagtatctttggcagtgtggccctggggcccgtgtgccctgctgtgtgcccgcctggcggtatccatcaggtcacagtcaatgaaagccttctggccccactcaatgtggagctggaccctgagatccagaaggtgcgcgcacaggagcgggagcagatcaaggctctgaacaa

SEQ ID NO: 44 - DNA, 223 bp, synthetic construct
  misc_feature 1..223: note = Krt71 Mt1
  source 1..223: mol_type = other DNA
atgagccgccaattcacctgcaagtctggagccagcaacaggggcttcagtggttgctccgcagtgctctctgggggaagctcatcctcctaccgggcaggaggcccggtatccatcaggtcacagtcaatgaaagccttctggccccactcaatgtggagctggaccctgagatccagaaggtgcgcgcacaggagcgggagcagatcaaggctctgaacaa

SEQ ID NO: 45 - DNA, 309 bp, synthetic construct
  misc_feature 1..309: note = Krt71 Mt2
  source 1..309: mol_type = other DNA
atgagccgccaattcacctgcaagtctggagccagcaacaggggcttcagtggttgctccgcagtgctctctgggggaagctcatcctcctaccgggcagcgggggctttggcagtcggagtctctacagcctgggaggtggcaggagcatcactcttaacatggctagtggcagcgggaagaacggaggggcggtatccatcaggtcacagtcaatgaaagccttctggccccactcaatgtggagctggaccctgagatccagaaggtgcgcgcacaggagcgggagcagatcaaggctctgaacaa

SEQ ID NO: 46 - DNA, 316 bp, synthetic construct
  misc_feature 1..316: note = Krt71 Mt3
  source 1..316: mol_type = other DNA
atgagccgccaattcacctgcaagtctggagccagcaacaggggcttcagtggttgctccgcagtgctctctgggggaagctcatcctcctaccgggcagggctcagcgggggctttggcagtcggagtctctacagcctgggaggtggcaggagcatcactcttaacatggctagtggcagcgggaagaacggaggggcggtatccatcaggtcacagtcaatgaaagccttctggccccactcaatgtggagctggaccctgagatccagaaggtgcgcgcacaggagcgggagcagatcaaggctctgaacaa

SEQ ID NO: 47 - DNA, 414 bp, synthetic construct
  misc_feature 1..414: note = Krt71 Mt4
  source 1..414: mol_type = other DNA
atgagccgccaattcacctgcaagtctggagccagcaacaggggcttcagtggttgctccgcagtgctctctgggggaagctcatcctcctaccgggcaggaggcaaagggctcagcgggggctttggcagtcggagtctctacagcctgggaggtggcaggagcatcactcttaacatggctagtggcagcgggaagaacggaggttttggatttggccggaaccgagccagtggctttgccggaagtatctttggcagtgtggccctggggcccgtgtgccctgctgtgtgcccgcggtatccatcaggtcacagtcaatgaaagccttctggccccactcaatgtggagctggaccctgagatccagaaggtgcgcgcacaggagcgggagcagatcaaggctctgaacaa

SEQ ID NO: 48 - DNA, 325 bp, synthetic construct
  misc_feature 1..325: note = Krt71 Mt5
  source 1..325: mol_type = other DNA
atgagccgccaattcacctgcaagtctggagccagcaacaggggcttcagtggttgctccgcagtgctctctgggggaagctcatcctcctaccgggcaggaggcaaagggctcagcgggggctttggcagtcggagtctctacagcctgggaggtggcaggagcatcactcttaacatggctagtggcagcgggaagaacggaggggcggtatccatcaggtcacagtcaatgaaagccttctggccccactcaatgtggagctggaccctgagatccagaaggtgcgcgcacaggagcgggagcagatcaaggctctgaacaa

SEQ ID NO: 49 - DNA, 400 bp, synthetic construct
  misc_feature 1..400: note = Krt71 Mt6
  source 1..400: mol_type = other DNA
atgagccgccaattcacctgcaagtctggagccagcaacaggggcttcagtggttgctccgcagtgctctctgggggaagctcatcctcctaccgggctcagcgggggctttggcagtcggagtctctacagcctgggaggtggcaggagcatcactcttaacatggctagtggcagcgggaagaacggaggttttggatttggccggaaccgagccagtggctttgccggaagtatctttggcagtgtggccctggggcccgtgtgccctgctgtgtgcccgcggtatccatcaggtcacagtcaatgaaagccttctggccccactcaatgtggagctggaccctgagatccagaaggtgcgcgcacaggagcgggagcagatcaaggctctgaacaa

SEQ ID NO: 50 - DNA, 405 bp, synthetic construct
  misc_feature 1..405: note = Krt71 Mt7
  source 1..405: mol_type = other DNA
atgagccgccaattcacctgcaagtctggagccagcaacaggggcttcagtggttgctccgcagtgctctctgggggaagctcatcctcctaccgggcagggctcagcgggggctttggcagtcggagtctctacagcctgggaggtggcaggagcatcactcttaacatggctagtggcagcgggaagaacggaggttttggatttggccggaaccgagccagtggctttgccggaagtatctttggcagtgtggccctggggcccgtgtgccctgctgtgtgcccgcggtatccatcaggtcacagtcaatgaaagccttctggccccactcaatgtggagctggaccctgagatccagaaggtgcgcgcacaggagcgggagcagatcaaggctctgaacaa

SEQ ID NO: 51 - DNA, 214 bp, synthetic construct
  misc_feature 1..214: note = Krt71 Mt8
  source 1..214: mol_type = other DNA
atgagccgccaattcacctgcaagtctggagccagcaacaggggcttcagtggttgctccgcagtgctctctgggggaagctcatcctcctaccgggcaggatccatcaggtcacagtcaatgaaagccttctggccccactcaatgtggagctggaccctgagatccagaaggtgcgcgcacaggagcgggagcagatcaaggctctgaacaa

SEQ ID NO: 52 - DNA, 352 bp, synthetic construct
  misc_feature 1..352: note = Krt71 Mt9
  source 1..352: mol_type = other DNA
atgagccgccaattcacctgcaagtctggagccagcaacaggggcttcagtggttgctccgcagtgctctctgggggaagctcatcctcctaccgggcatcactcttaacatggctagtggcagcgggaagaacggaggttttggatttggccggaaccgagccagtggctttgccggaagtatctttggcagtgtggccctggggcccgtgtgccctgctgtgtgcccgcctggcggtatccatcaggtcacagtcaatgaaagccttctggccccactcaatgtggagctggaccctgagatccagaaggtgcgcgcacaggagcgggagcagatcaaggctctgaacaa

SEQ ID NO: 53 - DNA, 418 bp, synthetic construct
  misc_feature 1..418: note = Krt71 Mt10
  source 1..418: mol_type = other DNA
atgagccgccaattcacctgcaagtctggagccagcaacaggggcttcagtggttgctccgcagtgctctctgggggaagctcatcctcctaccgggcaggaggcaaagggctcagcgggggctttggcagtcggagtctctacagcctgggaggtggcaggagcatcactcttaacatggctagtggcagcgggaagaacggaggttttggatttggccggaaccgagccagtggctttgccggaagtatctttggcagtgtggccctggggcccgtgtgccctgctgtgtgcccgcctgcggtatccatcaggtcacagtcaatgaaagccttctggccccactcaatgtggagctggaccctgagatccagaaggtgcgcgcacaggagcgggagcagatcaaggctctgaacaa

SEQ ID NO: 54 - DNA, 412 bp, synthetic construct
  misc_feature 1..412: note = Krt71 Mt11
  source 1..412: mol_type = other DNA
atgagccgccaattcacctgcaagtctggagccagcaacaggggcttcagtggttgctccgcagtgctctctgggggaagctcatcctcctaccgggcagaagggctcagcgggggctttggcagtcggagtctctacagcctgggaggtggcaggagcatcactcttaacatggctagtggcagcgggaagaacggaggttttggatttggccggaaccgagccagtggctttgccggaagtatctttggcagtgtggccctggggcccgtgtgccctgctgtgtgcccgcctgcggtatccatcaggtcacagtcaatgaaagccttctggccccactcaatgtggagctggaccctgagatccagaaggtgcgcgcacaggagcgggagcagatcaaggctctgaacaa

SEQ ID NO: 55 - DNA, 412 bp, synthetic construct
  misc_feature 1..412: note = Krt71 Mt12
  source 1..412: mol_type = other DNA
atgagccgccaattcacctgcaagtctggagccagcaacaggggcttcagtggttgctccgcagtgctctctgggggaagctcatcctcctaccgggcaggaaagggctcagcgggggctttggcagtcggagtctctacagcctgggaggtggcaggagcatcactcttaacatggctagtggcagcgggaagaacggaggttttggatttggccggaaccgagccagtggctttgccggaagtatctttggcagtgtggccctggggcccgtgtgccctgctgtgtgcccgccattcatccatcaggtcacagtcaatgaaagccttctggccccactcaatgtggagctggaccctgagatccagaaggtgcgcgcacaggagcgggagcagatcaaggctctgaacaa

SEQ ID NO: 56 - DNA, 415 bp, synthetic construct
  misc_feature 1..415: note = Krt71 Mt13
  source 1..415: mol_type = other DNA
atgagccgccaattcacctgcaagtctggagccagcaacaggggcttcagtggttgctccgcagtgctctctgggggaagctcatcctcctaccgggcaggaaagggctcagcgggggctttggcagtcggagtctctacagcctgggaggtggcaggagcatcactcttaacatggctagtggcagcgggaagaacggaggttttggatttggccggaaccgagccagtggctttgccggaagtatctttggcagtgtggccctggggcccgtgtgccctgctgtgtgcccgcctggcggtatccatcaggtcacagtcaatgaaagccttctggccccactcaatgtggagctggaccctgagatccagaaggtgcgcgcacaggagcgggagcagatcaaggctctgaacaa

SEQ ID NO: 57 - DNA, 418 bp, synthetic construct
  misc_feature 1..418: note = Krt72 WT
  source 1..418: mol_type = other DNA
atgagccgccagttgaccctctatcccggagctgagcgcctgggtttcagtggctgctctgcggtcatctcaggcaggctcagtggcagtcacgcctcggtccgagctggagtcaagggagcagcatttgggagcagaagcctgttctgtgtggggggaggccggcggctggcgttgagctctgcagggcgaagtggtggcttcacgctgggccacggaggggcgagcggtgggcggcctgggggcttcgtgggcaccgtcttcggcagcgcgggactggggcccacatgcccatcagtgtgccctcccggtggcatcccccaggttgtcgtcaacaagagccttctggccccactcaatgtggagctggacccggagatccagaaggtgcgggcacaagagagggagcagatcaagg

SEQ ID NO: 58 - DNA, 395 bp, synthetic construct
  misc_feature 1..395: note = Krt72Mt1
  source 1..395: mol_type = other DNA
atgaccctctatcccggagctgagcgcctgggtttcagtggctgctctgcggtcatctcaggcagtcacgcctcggtccgagctggagtcaagggagcagcatttgggagcagaagcctgttctgtgttggggggaggccggcggctggcgttgagctctgcagggcgaagtggtggcttcacgctgggccacggaggggcgagcggtgggcggcctgggggcttcgtgggcaccgtcttcggcagcgcgggactggggcccacatgcccatcagtgtgccctcccggtggcatcccccaggttgtcgtcaacaagagccttctggccccactcaatgtggagctggacccggagatccagaaggtgcgggcacaagagagggagcagatcaagg

SEQ ID NO: 59 - DNA, 332 bp, synthetic construct
  misc_feature 1..332: note = Krt72Mt2
  source 1..332: mol_type = other DNA
atgagccgcctcggtccgagctggagtcaagggagcagcatttgggagcagaagcctgttctgtgtggggggaggccggcggctggcgttgagctctgcagggcgaagtggtggcttcacgctgggccacggaggggcgagcggtgggcggcctgggggcttcgtgggcaccgtcttcggcagcgcgggactggggcccacatgcccatcagtgtgccctcccggtggcatcccccaggttgtcgtcaacaagagccttctggccccactcaatgtggagctggacccggagatccagaaggtgcgggcacaagagagggagcagatcaagg

SEQ ID NO: 60 - DNA, 396 bp, synthetic construct
  misc_feature 1..396: note = Krt72Mt3
  source 1..396: mol_type = other DNA
atgaccctctatcccggagctgagcgcctgggtttcagtggctgctctgcggtcatctcagtggcagtcacgcctcggtccgagctggagtcaagggagcagcatttgggagcagaagcctgttctgtgtggggggaggccggcggctggcgttgagctctgcagggcgaagtggtggcttcacgctgggccacggaggggcgagcggtgggcggcctgggggcttcgtgggcaccgtcttcggcagcgcgggactggggcccacatgcccatcagtgtgccctcccggtggcatcccccaggttgtcgtcaacaagagccttctggccccactcaatgtggagctggacccggagatccagaaggtgcgggcacaagagagggagcagatcaagg

SEQ ID NO: 61 - DNA, 392 bp, synthetic construct
  misc_feature 1..392: note = Krt72Mt4
  source 1..392: mol_type = other DNA
atgaccctctatcccggagctgagcgcctgggtttcagtggctgctctgcggtcatctcaggcagtcacgcctcggtccgagctggagtcaagggagcagcatttgggagcagaagcctgttctgtggggggaggccggcggctggcgttgagctctgcagggcgaagtggtggcttcacgctgggccacggaggggcgagcggtgggcggcctgggggcttcgtgggcaccgtcttcggcagcgcgggactggggcccacatgcccatcagtgtgccctcccggtggcatcccccaggttgtcgtcaacaagagccttctggccccactcaatgtggagctggacccggagatccagaaggtgcgggcacaagagagggagcagatcaagg

SEQ ID NO: 62 - DNA, 261 bp, synthetic construct
  misc_feature 1..261: note = Krt72Mt5
  source 1..261: mol_type = other DNA
atgagccgcggctggcgttgagctctgcagggcgaagtggtggcttcacgctgggccacggaggggcgagcggtgggcggcctgggggcttcgtgggcaccgtcttcggcagcgcgggactggggcccacatgcccatcagtgtgccctcccggtggcatcccccaggttgtcgtcaacaagagccttctggccccactcaatgtggagctggacccggagatccagaaggtgcgggcacaagagagggagcagatcaagg

SEQ ID NO: 63 - DNA, 390 bp, synthetic construct
  misc_feature 1..390: note = Krt72Mt6
  source 1..390: mol_type = other DNA
atgagccgcctgggtttcagtggctgctctgcggtcatctcaggcaggctcagtggcagtcacgcctcggtccgagctggagtcaagggagcagcatttgggagcagaagcctgttctgtgttgggggggaggccggcggctggcgttgagctctgcagggcgaagtggtggcttcacgctgggccacggaggggcgagcggtgggcggcctgggggcttcgtgggcaccgtcttcggcagcgcgggactggggcccacatgcccatcagtgtgccctcccggtggcatcccccaggttgtcgtcaacaagagccttctggccccactcaatgtggagctggacccggagatccagaaggtgcgggcacaagagagggagcagatcaagg

SEQ ID NO: 64 - DNA, 420 bp, synthetic construct
  misc_feature 1..420: note = Krt72Mt7
  source 1..420: mol_type = other DNA
atgagccgccaagttgaccctctatcccggagctgagcgcctgggtttcagtggctgctctgcggtcatctcaggcaggctcagtggcagtcacgcctcggtccgagctggagtcaagggagcagcatttgggagcagaagcctgttctgtgttggggggaggccggcggctggcgttgagctctgcagggcgaagtggtggcttcacgctgggccacggaggggcgagcggtgggcggcctgggggcttcgtgggcaccgtcttcggcagcgcgggactggggcccacatgcccatcagtgtgccctcccggtggcatcccccaggttgtcgtcaacaagagccttctggccccactcaatgtggagctggacccggagatccagaaggtgcgggcacaagagagggagcagatcaagg

SEQ ID NO: 65 - DNA, 341 bp, synthetic construct
  misc_feature 1..341: note = Krt72Mt8
  source 1..341: mol_type = other DNA
atgagccgcagtcacgcctcggtccgagctggagtcaagggagcagcatttgggagcagaagcctgttctgtgttggggggaggccggcggctggcgttgagctctgcagggcgaagtggtggcttcacgctgggccacggaggggcgagcggtgggcggcctgggggcttcgtgggcaccgtcttcggcagcgcgggactggggcccacatgcccatcagtgtgccctcccggtggcatcccccaggttgtcgtcaacaagagccttctggccccactcaatgtggagctggacccggagatccagaaggtgcgggcacaagagagggagcagatcaagg

SEQ ID NO: 66 - DNA, 278 bp, synthetic construct
  misc_feature 1..278: note = Krt72Mt9
  source 1..278: mol_type = other DNA
atgagccgccatggggggaggccggcggctggcgttgagctctgcagggcgaagtggtggcttcacgctgggccacggaggggcgagcggtgggcggcctgggggcttcgtgggcaccgtcttcggcagcgcgggactggggcccacatgcccatcagtgtgccctcccggtggcatcccccaggttgtcgtcaacaagagccttctggccccactcaatgtggagctggacccggagatccagaaggtgcgggcacaagagagggagcagatcaagg

SEQ ID NO: 67 - DNA, 411 bp, synthetic construct
  misc_feature 1..411: note = Krt72Mt10
  source 1..411: mol_type = other DNA
atgagccgccaagttgaccctctatcccggagctgagcgcctgggtttcagtggctgctctgcggtcatctcaggcaggctcagtggcagtcacgcctcggtccgagctggagtcaagggagcagcatttgggagcagaagctcatttgggaggccggcggctggcgttgagctctgcagggcgaagtggtggcttcacgctgggccacggaggggcgagcggtgggcggcctgggggcttcgtgggcaccgtcttcggcagcgcgggactggggcccacatgcccatcagtgtgccctcccggtggcatcccccaggttgtcgtcaacaagagccttctggccccactcaatgtggagctggacccggagatccagaaggtgcgggcacaagagagggagcagatcaagg

SEQ ID NO: 68 - DNA, 428 bp, synthetic construct
  misc_feature 1..428: note = Krt73WT
  source 1..428: mol_type = other DNA
atgaatcgccaattcacctgcaaacctggagttgccaacaggggcttcagcggctgctcagctgtgctctccggaggcagctcatcctcttaccgggcagccggcaaagggctcagtggaggcttcagcagtcggagcctctacagcctgaggagtcccaggagcatctccttcaatgtggctagcagcagcgggcgcacagggggatatgggtttggccggaatcgggccagtggctttgctggcagtatgtttggcagtggggctctggggccttcaaatccatccttgtgcctgcctggaggcatccaccaggtaacagtcaataaaagcctcctggctcctctcaatgtggagctggacccggagatccagaaggtgcgcgcccaggagcgggagcagatcaaggctctgaacaacaaattcgc

SEQ ID NO: 69 - DNA, 408 bp, synthetic construct
  misc_feature 1..408: note = Krt73Mt1
  source 1..408: mol_type = other DNA
atgaatcgccaattcacctgcaaacctggagttgccaacaggggcttcagcggctgctcagctgtgctctccggaggcagctcatcctcttaccgggcagggctcagtggaggcttcagcagtcggagcctctacagcctgaggagtcccaggagcatctccttcaatgtggctagcagcagcgggcgcacagggggatatgggtttggccggaatcgggccagtggctttgctggcagtatgtttggcagtggggctctggggccttcaaatccatccttgaggcatccaccaggtaacagtcaataaaagcctcctggctcctctcaatgtggagctggacccggagatccagaaggtgcgcgcccaggagcgggagcagatcaaggctctgaacaacaaattcgc

SEQ ID NO: 70 - DNA, 237 bp, synthetic construct
  misc_feature 1..237: note = Krt73Mt2
  source 1..237: mol_type = other DNA
atgaatcgccaattcacctgcaaacctggagttgccaacaggggcttcagcggctgctcagctgtgctctccggaggcagctcatcctcttaccgggcagccggtgcctggaggcatccaccaggtaacagtcaataaaagcctcctggctcctctcaatgtggagctggacccggagatccagaaggtgcgcgcccaggagcgggagcagatcaaggctctgaacaacaaattcgc

SEQ ID NO: 71 - DNA, 317 bp, synthetic construct
  misc_feature 1..317: note = Krt73Mt3
  source 1..317: mol_type = other DNA
atgaatcgccaattcacctgcaaacctggagttgccaacaggggcttcagcggctgctcagctgtgctctccggaggcagctcatcctcttaccgggcagctcagtggaggcttcagcagtcggagcctctacagcctgaggagtcccaggagcatctccttcaatgtggctagcagcagcgggcgcacagaggcatccaccaggtaacagtcaataaaagcctcctggctcctctcaatgtggagctggacccggagatccagaaggtgcgcgcccaggagcgggagcagatcaaggctctgaacaacaaattcgc

SEQ ID NO: 72 - DNA, 424 bp, synthetic construct
  misc_feature 1..424: note = Krt73Mt4
  source 1..424: mol_type = other DNA
atgaatcgccaattcacctgcaaacctggagttgccaacaggggcttcagcggctgctcagctgtgctctccggaggcagctcatcctcttaccgggcagccggcaaagggctcagtggaggcttcagcagtcggagcctctacagcctgaggagtcccaggagcatctccttcaatgtggctagcagcagcgggcgcacagggggatatgggtttggccggaatcgggccagtggctttgctggcagtatgtttggcagtggggctctggggccttcaaatccatccttgtgcctggaggcatccaccaggtaacagtcaataaaagcctcctggctcctctcaatgtggagctggacccggagatccagaaggtgcgcgcccaggagcgggagcagatcaaggctctgaacaacaaattcgc

SEQ ID NO: 73 - DNA, 424 bp, synthetic construct
  misc_feature 1..424: note = Krt73Mt5
  source 1..424: mol_type = other DNA
atgaatcgccaattcacctgcaaacctggagttgccaacaggggcttcagcggctgctcagctgtgctctccggaggcagctcatcctcttaccgggcagccggaaaagggctcagtggaggcttcagcagtcggagcctctacagcctgaggagtcccaggagcatctccttcaatgtggctagcagcagcgggcgcacagggggatatgggtttggccggaatcgggccagtggctttgctggcagtatgtttggcagtggggctctggggccttcaaatccatccttgtgcctggaggcatccaccaggtaacagtcaataaaagcctcctggctcctctcaatgtggagctggacccggagatccagaaggtgcgcgcccaggagcgggagcagatcaaggctctgaacaacaaattcgc

SEQ ID NO: 74 - DNA, 328 bp, synthetic construct
  misc_feature 1..328: note = Krt73Mt6
  source 1..328: mol_type = other DNA
atgaatcgccaattcacctgcaaacctggagttgccaacaggggcttcagcggctgctcagctgtgctctccggaggcagctcatcctcttaccgggcagccggcaaagggctcagtggaggcttcagcagtcggagcctctacagcctgaggagtcccaggagcatctccttcaatgtggctagcagcagcgggcgcacagaggcatccaccaggtaacagtcaataaaagcctcctggctcctctcaatgtggagctggacccggagatccagaaggtgcgcgcccaggagcgggagcagatcaaggctctgaacaacaaattcgc

SEQ ID NO: 75 - DNA, 413 bp, synthetic construct
  misc_feature 1..413: note = Krt73Mt7
  source 1..413: mol_type = other DNA
atgaatcgccaattcacctgcaaacctggagttgccaacaggggcttcagcggctgctcagctgtgctctccggaggcagctcatcctcttaccgggcagctcagtggaggcttcagcagtcggagcctctacagcctgaggagtcccaggagcatctccttcaatgtggctagcagcagcgggcgcacagggggatatgggtttggccggaatcgggccagtggctttgctggcagtatgtttggcagtggggctctggggccttcaaatccatccttgtgcctggaggcatccaccaggtaacagtcaataaaagcctcctggctcctctcaatgtggagctggacccggagatccagaaggtgcgcgcccaggagcgggagcagatcaaggctctgaacaacaaattcgc

SEQ ID NO: 76 - DNA, 349 bp, synthetic construct
  misc_feature 1..349: note = Krt74WT
  source 1..349: mol_type = other DNA
atggcttcttgccacacagctggccacaggactggcctcagcagcaggagcctctacagtcttggagggaatcagcatacttcctacaatgtggcaggtggcagtgctcggggcacaaggcacagctttggatatgggtatggtgggggtcgagggagtggctttgccaacagcatgtttggcagcatggccctgggggccaattgtccatctgtgtgtctgtctgggggcatctaccaggtcacagtcaacaagagcctcctggctcccttgaatgtggagctggaccctgagatccagaaagtgcgtgcacaggagcgggagcagatcaaggctctgaacgacaagt

SEQ ID NO: 77 - DNA, 171 bp, synthetic construct
  misc_feature 1..171: note = Krt74Mt1
  source 1..171: mol_type = other DNA
atggcttcttgccacacagctggccacaggactggcctcagcagcaggagcctctataccaggtcacagtcaacaagagcctcctggctcccttgaatgtggagctggaccctgagatccagaaagtgcgtgcacaggagcgggagcagatcaaggctctgaacgacaagt

SEQ ID NO: 78 - DNA, 171 bp, synthetic construct; identical to SEQ ID NO: 77
  misc_feature 1..171: note = Krt74Mt2
  source 1..171: mol_type = other DNA

SEQ ID NO: 79 - DNA, 267 bp, synthetic construct
  misc_feature 1..267: note = Krt74Mt3
  source 1..267: mol_type = other DNA
atggcttcttgccacacagctggccacaggactggcctcagcagcaggagcctctatggtgggggtcgagggagtggctttgccaacagcatgtttggcagcatggccctgggggccaattgtccatctgtgtgtctgtctgggggcatctttaccaggtcacagtcaacaagagcctcctggctcccttgaatgtggagctggaccctgagatccagaaagtgcgtgcacaggagcgggagcagatcaaggctctgaacgacaagt

SEQ ID NO: 80 - DNA, 351 bp, synthetic construct
  misc_feature 1..351: note = Krt74Mt4
  source 1..351: mol_type = other DNA
atggcttcttgccacacagctggccacaggactggcctcagcagcaggagcctctaacagtcttggagggaatcagcatacttcctacaatgtggcaggtggcagtgctcggggcacaaggcacagctttggatatgggtatggtgggggtcgagggagtggctttgccaacagcatgtttggcagcatggccctgggggccaattgtccatctgtgtgtctgtctgggggcatcttaccaggtcacagtcaacaagagcctcctggctcccttgaatgtggagctggaccctgagatccagaaagtgcgtgcacaggagcgggagcagatcaaggctctgaacgacaagt

SEQ ID NO: 81 - DNA, 255 bp, synthetic construct
  misc_feature 1..255: note = Krt74Mt5
  source 1..255: mol_type = other DNA
atggcttcttgccacacagctggccacaggactggcctcagcagcaggagcctctacagtcttggagggaatcagcatacttcctacaatgtggcaggtggcagtgctcggggcacaaggcacagctttggatatgggtaaaccaggtcacagtcaacaagagcctcctggctcccttgaatgtggagctggaccctgagatccagaaagtgcgtgcacaggagcgggagcagatcaaggctctgaacgacaagt

SEQ ID NO: 82 - DNA, 171 bp, synthetic construct; identical to SEQ ID NO: 77
  misc_feature 1..171: note = Krt74Mt6
  source 1..171: mol_type = other DNA

SEQ ID NO: 83 - DNA, 186 bp, synthetic construct
  misc_feature 1..186: note = KAP8-1WT
  source 1..186: mol_type = other DNA
atgtactacaccggcgctgagggctctgtcttcccaggatgctactggggcagctatggctaccctctggggtacagtgttggctgtggctatggtagcacctactctccagttggctatggccttggctatggctacaatggctgcggggcttacagaagatactggccatttgctctctactga

SEQ ID NO: 84 - DNA, 134 bp, synthetic construct
  misc_feature 1..134: note = KAP8-1Mt1
  source 1..134: mol_type = other DNA
atgtactacaccggcgctgagggctctgtcttcccaggatgctatggctaccctctggagttggctatggccttggctatggctacaatggctgcggggcttacagaagatactggccatttgctctctactga

SEQ ID NO: 85 - DNA, 139 bp, synthetic construct
  misc_feature 1..139: note = KAP8-1Mt2
  source 1..139: mol_type = other DNA
atgtactacaccggcgctgagggctctgtcttcccaggatgctagggtacagtgttggctgtggctatggtagcaccttggctatggctacaatggctgcggggcttacagaagatactggccatttgctctctactga

SEQ ID NO: 86 - DNA, 137 bp, synthetic construct
  misc_feature 1..137: note = KAP8-1Mt3
  source 1..137: mol_type = other DNA
atgtactacaccggcgctgagggctctgtcttcccaggctgtggctatggtagcacctacttgttggctatggccttggctatggctacaatggctgcggggcttacagaagatactggccatttgctctctactga

SEQ ID NO: 87 - DNA, 73 bp, synthetic construct
  misc_feature 1..73: note = KAP8-1Mt4
  source 1..73: mol_type = other DNA
atgtactagccttggctatggctacaatggctgcggggcttacagaagatactggccatttgctctctactga

SEQ ID NO: 88 - DNA, 189 bp, synthetic construct
  misc_feature 1..189: note = KAP8-2WT
  source 1..189: mol_type = other DNA
atgagctactacggcagctactacggaggtctgggctctggcatccgaggctttgggaacctgggttatggctatggctgtggctgtggctttggaggttacggatatggatctggctatggcagatatggatatggctaccgccgccccctttattatggaggatatggattctcccgattctactga

SEQ ID NO: 89 - DNA, 130 bp, synthetic construct
  misc_feature 1..130: note = KAP8-2Mt1
  source 1..130: mol_type = other DNA
atgagctactacggcagctactacggaggtctgggctctggcatccgaggcatctggctatggcagatatggatatggctaccgccgccccctttattatggaggatatggattctcccgattctactga

SEQ ID NO: 90 - DNA, 190 bp, synthetic construct
  misc_feature 1..190: note = KAP8-2Mt2
  source 1..190: mol_type = other DNA
atgagctactacggcagctactacggaggtctgggctctggcatccgaggctttgggaacctgggttatggctatggctgtggctgtggctttggaggttacggatatgggatctggctatggcagatatggatatggctaccgccgccccctttattatggaggatatggattctcccgattctactga

SEQ ID NO: 91 - DNA, 83 bp, synthetic construct
  misc_feature 1..83: note = KAP8-2Mt3
  source 1..83: mol_type = other DNA
atgaatctggctatggcagatatggatatggctaccgccgccccctttattatggaggatatggattctcccgattctactga

SEQ ID NO: 92 - DNA, 187 bp, synthetic construct
  misc_feature 1..187: note = KAP8-2Mt4
  source 1..187: mol_type = other DNA
atgagctactacggcagctactacggaggtctgggctctggcatccgaggctttgggaacctgggttatggctatggctgtggctgtggctttggaggttacggatatatctggctatggcagatatggatatggctaccgccgccccctttattatggaggatatggattctcccgattctactga

SEQ ID NO: 93 - DNA, 232 bp, synthetic construct
  misc_feature 1..232: note = Tyr WT
  source 1..232: mol_type = other DNA
gagcctgtgcctcctctaagaacttgttggcaaaagaatgctgcccaccatggatgggtgatgggagtccctgcggccagctttcaggcagaggttcctgccaggatatccttctgtccagtgcaccatctggacctcagttccccttcaaaggggtggatgaccgtgagtcctggccctctgtgttttataataggacctgccagtgctcaggcaacttcatgggtttcaa

SEQ ID NO: 94 - DNA, 142 bp, synthetic construct
  misc_feature 1..142: note = Tyr Mt1
  source 1..142: mol_type = other DNA
gagcctgtgcagcaaaagaatgctgcccaccatggatgggtgatgggagtccctgcggccagctttcaggcagaggttcctgccaggatatccttctgtccagtgcaccatctggacctcagttccccttcatgggtttcaa

SEQ ID NO: 95 - DNA, 233 bp, synthetic construct
  misc_feature 1..233: note = Fgf5 WT
  source 1..233: mol_type = other DNA
tgcagccacctgatccacagcgcttgggctcacggggagaagcgtctcactcccgaagggcaacccgcgcctcctaggaacccgggagactccagcggcagccggggcagaagtagcgcgacgttttcttcgtcttctgcctcctcaccagtcgcagcttctccgggcagccaaggaagcggctcggaacatagcagtttccagtggagcccttcggggcgccggaccggcag

SEQ ID NO: 96 - DNA, 144 bp, synthetic construct
  misc_feature 1..144: note = Fgf5 Mt1
  source 1..144: mol_type = other DNA
tgcagccacccgggagactccagcggcagccggaagtagcgcgacgttttcttcgtcttctgcctcctcaccagtcgcagcttctccgggcagccaaggaagcggctcggaacatagcagtttccagtggagccggaccggcag

SEQ ID NO: 97 - RNA, 20 nt, synthetic construct
  misc_feature 1..20: note = gKAP8-1 crRNA1
  source 1..20: mol_type = other RNA
gcaacctgggaagacggtgc

SEQ ID NO: 98 - RNA, 20 nt, synthetic construct
  misc_feature 1..20: note = gKAP8-1 crRNA2
  source 1..20: mol_type = other RNA
tacagtgtgggctgtggcta

SEQ ID NO: 99 - RNA, 20 nt, synthetic construct
  misc_feature 1..20: note = gKAP8-1 crRNA3
  source 1..20: mol_type = other RNA
cggtagtacctactccccag

SEQ ID NO: 100 - DNA, 100 bp, synthetic construct
  misc_feature 1..100: note = Cas9 EP enhancer
  source 1..100: mol_type = other DNA
ttagctctgtttacgtcccagcgggcatgagagtaacaagagggtgtggtaatattacggtaccgagcactatcgatacaatatgtgtcatacggacacg

SEQ ID NO: 101 - DNA, 24 bp, synthetic construct
  misc_feature 1..24: note = gKrtap8-1-Fw3
  source 1..24: mol_type = other DNA
ttggggtcaagaatgaaaatgacg

SEQ ID NO: 102 - DNA, 20 bp, synthetic construct
  misc_feature 1..20: note = gKrtap8-1-Rv3
  source 1..20: mol_type = other DNA
aacatcatgcagggaaggca

SEQ ID NO: 103 - DNA, 56 bp, synthetic construct
  misc_feature 1..56: note = gKAP8-1_Miseq_Fw
  source 1..56: mol_type = other DNA
tcgtcggcagcgtcagatgtgtataagagacagcccgggtatataaagaagggagc

SEQ ID NO: 104 - DNA, 54 bp, synthetic construct
  misc_feature 1..54: note = gKAP8-1_Miseq_Rv
  source 1..54: mol_type = other DNA
gtctcgtgggctcggagatgtgtataagagacagaacatcatgcagggaaggca

SEQ ID NO: 105 - DNA, 189 bp, synthetic construct
  misc_feature 1..189: note = gKAP8-1WT
  source 1..189: mol_type = other DNA
atgagctactgcttctccagcaccgtcttcccaggttgctactggggcagctatggctaccctctgggctacagtgtgggctgtggctacggtagtacctactccccagtgggctatggcttcggctatggctacaacggctctggggccttcggttgccgaagattctggccatttgcgctctactga

SEQ ID NO: 106 - DNA, 183 bp, synthetic construct
  misc_feature 1..183: note = gKAP8-1Mt1
  source 1..183: mol_type = other DNA
atgagctactgcttctccagcaccgtcttcccaggttgctactggggcagctatggctaccctctgggctacagtgtgggctgtggtagtacctactccccagtgggctatggcttcggctatggctacaacggctctggggccttcggttgccgaagattctggccatttgcgctctactga

SEQ ID NO: 107 - DNA, 53 bp, synthetic construct
  misc_feature 1..53: note = Krt72-Miseq_Fw
  source 1..53: mol_type = other DNA
tcgtcggcagcgtcagatgtgtataagagacagccaggagtgcagctgtatcc

SEQ ID NO: 108 - DNA, 54 bp, synthetic construct
  misc_feature 1..54: note = Krt72-Miseq_Rv
  source 1..54: mol_type = other DNA
gtctcgtgggctcggagatgtgtataagagacagacattgagtggggccagaag